European Patent Specification EP 3 976 835 B1, published July 17, 2024. Title: A method for determining a yeast having extracellular glucoamylase STA1p activity in a sample and tools and uses related thereto. Applicant: Teknologian tutkimuskeskus VTT Oy. The sequence listing filed with the application follows.

SEQUENCE LISTING (27 sequences)

SEQ ID NO: 1 - DNA, 5225 bp, Saccharomyces cerevisiae
ggaatgaacagcgccaagtagcactggacaaactgcagaaagtattagtacttgctttattccgtgtatcgtactttaggtcgtcagttttacacttcggtacgcaaatgaaaataaaaagctcattcacaacttagacacaatttcgccatttacaagtagctgaagagtccatctatcgaattatgaatgatgctattttaaatatcgtcgttgctgcactcgttttccatgttctttttatccacacatccgatgttttatttacagttgagcatctcagggccagcgacaaatataaacatattatactcaaaatgaagctcgttgaaaagaggatatttcttaacctcttttacagtgttttcaacaccttttcatctgtgtgccatgtcagattaaggatgctcaacttttcgaattattattacaaatttcaaagaaattactattcctttttgtcccctaatgtatccctcatttcataccgtcgttttggggttccaactgcacatagctttcaagtgtggttttacggtaagaacaacccccccatcggttggtgcggaatactttcctattctcatcgagagccgagccatacacctaaggtggacagaaagctaaaattccaaaacagaaaaatctaacatctttgctcccttacaagtaggaacgctagcgtatcaacccatctccagatttgcccagcatttctgtagaacacccaatgcgaatgaagactaatgaatattttaaaggcaaaaaataggaaaagtttaattattgatggttctcaccaccgcaaaacggtcacttgcatgcattgaggacatgcatctgcagtacttgtttttctcgaatgttttttaccatctcttttttccttatctgagctgctgacgcagacggacattgtttcatatttcgaaagctgtgcgggaaaacggacccaaacacgaatgtggatgcgctaatcggtatttccatctcatgaaacctgctactttttcagtgctcttcgtatgcatttcccaaaattcattcgtagccttgtcaacttagactcagttccacggcgtgcaggacggggtattatgaataaaggatccacgggtaagatttgttctatgttttaggtatggagttttgtaccacaaaactttaggaataccggattgtgtgcctacgccagccccagagtatgttctcacggctgtaattcctagtgatcttttcctggctcaaattaaactttcgcggcaggaaaaaaaaggctttttcttttttgtgtttcagtttctcggaatgtggcattacataagcataatcctttttgggtgtgcctggaaagttcaaattaagggttttttcttttgttttcttgacaagaaaatgttgcccaaagagtttcggccgttattttcctatccaagtgggtcctttttgtctttagtccttctctggggctagcgatcgctgcaaaattaggcttcactggtacgagttaactttttttctttttttttgtcatccttttctttggggctaaaaatggacttcccttttctttttctttgttgcagcagtggcttcaaagaactgctgattgctcaaggcaatcagttaaaagaaaaattagctttttttgtcaggcattgcacaaacttttttatttctgcctatactcttagacagatcagtcattcatgttgtctttttaacggtcgtactgggacatcgcataccttgagattccgtaattaggtgcaacaatacgggcacaactcattctgcggtatcttcacggacagaatttctattgcctattggtggtgtgattaacaattggaagcgcagagcttagaatggattttcaattcaatggatttggaggtattcgtttgtttactaatatttactttgaggacattgcccaaccctaaaagtgcctgttccagaacagaataacattatgatacgttttcctgaccgctgagcaatttaaagcaattagtagggtacgattgtttctagagaaatgtgggtcatctttttaggtccgttctcttctgatgaggtaacctttacaaaaatgtcatggagttaccaattgggattcaaggcatcatcacaatatacttcgttcttttacggagaaattaagctctttctactttgaattaactgttagacttgtcttatctgagaaatgtccgtgttcaaattaaataaaaatttagggcagttttatttaccttaacaaatatgttcaagcatttacgttactgcgctctcttctagttcaagaacggataactcatagacttacctgtacaagttgttgaagggttctcaattgataaaaaaggatcttttgcttcctaaactaaacctataaaaagcaccctattcatcagttataatctcttgtcatgttgtggttctaattgaaaatatactttggtaggcctcaaaaatccatatacgcacactatgcaaagaccatttctacttgcttatttggtcctttcgcttctatttaactcagctttgggttttccaactgcactagttcctagaggatcctcctctagcaacatcacttcctccggtccatcttcaactccattcagctctgctactgaaagcttttctactggcactactgtcactccatcatcatccaaataccctggcagtaaaacagaaacttctgtttcttctacaaccgaaactaccattgttccaactacaactacgacttctgtcataacaccatcaacaaccactattaccactacggtttgctctacaggaacaaactctgccggtgaaactacttctggatgctctccaaagaccattacaactactgttccatgttcaaccagtccaagcgaaaccgcatcggaatcaacaaccacttcacctaccacacctgtaactacagttgtctcaaccaccgtcgttactactgagtattctactagtacaaaacaaggtggtgaaattacaactacatttgtcaccaaaaacattccaaccacttacctaactacaattgctccaacttcatcagtcactacggttaccaatttcaccccaaccactattactactacggtttgctctacaggaacaaactctgccggtgaaactacctctggatgctctccaaagactgtcacaacaactgttccttgttcaactggtactggcgaatacactactgaaactaccgcccctgttacaacagctgtcacaaccaccgttgttaccactgaatcctctacgggtactaactccgctggtaagacgacaactagttacacaacaaagtctgtaccaaccacctatgtatttgactttggcaagggcattctcgatcaaagctgcggcggtgtattttcaaacaacggctctttgcaagtgcagctgcgggatgcagtcttgatgaatgggacagtggtatacgattcaaacggcgcttgggacagtagtgcgctggaggagtggctccagcgacagaaaaaagtttccatcgaaagaatatttgaaaatattgggcccagcgccgtgtatccgtctattttgcctggggtcgtgattgcgtcaccatcgcaaacgcatccagactacttctaccaatggataagggacagcgcgttgacgataaacagtattgtctctcattctgcggacccggcaatagagacgttattgcagtacctgaacgtttcattccacttgcaaagaaccaacaacacattgggcgctggcattggttacactaacgatacagtggctttgggagaccctaagtggaacgtcgacaacacggctttcacggaaccttggggtcgtcctcaaaacgatggccctgctcttcgaagcattgccatcttaaaaatcatcgactacatcaagcaatctggcactgatctgggggccaagtacccattccagtccaccgcagatatctttgatgatattgtacgttgggacctgaggttcattattgaccactggaattcttccggatttgatctatgggaggaagtcaatggcatgcatttctttactttactggtacaactgtctgcagtggacagatcgctgtcgtattttaacgcctcagaacggtcgtctccctttgttgaagaattgcgtcagacacgccgggacatctccaagtttttagtggaccctgcgaatgggtttatcaacggcaagtacaattatattgttgagacacccatgattgccgacacattgagatccggactggacatatccactttattagctgcgaacaccgtccacgatgcgccatctgcttcccatcttccgttcgatatcaatgaccctgccgtcctgaacacgttgcaccatttgatgttgcacatgcgttcgatataccccatcaacgatagctccaaaaatgcaacgggtattgccctgggccggtatcctgaggacgtatatgatggatatggctttggcgagggaaatccctgggtcctggccacgtgtgccgcttcaacaacgctttatcagctcatttacagacacatctctgagcagcatgacttggttgtcccaatgaacaacgattgttcgaacgcattttggagcgagctggtattctccaacctcacgactttgggaaatgacgaaggctatttgattttggagttcaatacacctgccttcaatcaaaccatacaaaaaatcttccaactagctgattcattcttggtcaagctgaaagctcacgtgggaacagacggggaactaagtgaacaatttaacaaatacacagggtttatgcagggtgcccaacaccttacctggtcctatacttcattctgggatgcctatcaaataagacaagaagttttacagagtttgtagacaaaaaaaaataaaagaaaagcgagaagtatacacaagtgtatttcctagatatttacatcaaatatatatatatatacttatttacaaaactctgatattataaattagttagatactatgtcggaacgtccagcccaaccacgtttgcagttcttttcactttctcatcctgtgtcaacttgttgccaggattgtatctgtcgaccagctcctcgtattctctttggttgtccaagaacttgatgatgtccaaagcgtgttcgaatatctcgtcaacgttttgtccctgggccacctttttctcc

SEQ ID NO: 2 - DNA, 22 bp, Artificial Sequence
  oligonucleotide
cctggctcaaattaaactttcg

SEQ ID NO: 3 - DNA, 21 bp, Artificial Sequence
  oligonucleotide
accaccaataggcaatagaaa

SEQ ID NO: 4 - DNA, 20 bp, Artificial Sequence
  oligonucleotide
caaggcaatcagttaaaaga

SEQ ID NO: 5 - DNA, 20 bp, Artificial Sequence
  oligonucleotide
caactacgacttctgtcata

SEQ ID NO: 6 - DNA, 19 bp, Artificial Sequence
  oligonucleotide
gatggtgacgcaatcacga

SEQ ID NO: 7 - DNA, 20 bp, Artificial Sequence
  oligonucleotide
tggaatgaacagcgccaagt

SEQ ID NO: 8 - DNA, 20 bp, Artificial Sequence
  oligonucleotide
agtgggagaaaaaggtggcc

SEQ ID NO: 9 - DNA, 20 bp, Artificial Sequence
  oligonucleotide
aatgaacagcgccaagtagc

SEQ ID NO: 10 - DNA, 21 bp, Artificial Sequence
  oligonucleotide
ttgaaagctatgtgcagttgg

SEQ ID NO: 11 - DNA, 21 bp, Artificial Sequence
  oligonucleotide
tgtcccctaatgtatccctca

SEQ ID NO: 12 - DNA, 22 bp, Artificial Sequence
  oligonucleotide
aaatcttacccgtggatccttt

SEQ ID NO: 13 - DNA, 20 bp, Artificial Sequence
  oligonucleotide
cccaaaattcattcgtagcc

SEQ ID NO: 14 - DNA, 20 bp, Artificial Sequence
  oligonucleotide
tatgcgatgtcccagtacga

SEQ ID NO: 15 - DNA, 20 bp, Artificial Sequence
  oligonucleotide
tgtcaggcattgcacaaact

SEQ ID NO: 16 - DNA, 21 bp, Artificial Sequence
  oligonucleotide
caattgagaacccttcaacaa

SEQ ID NO: 17 - DNA, 24 bp, Artificial Sequence
  oligonucleotide
agggcagttttatttaccttaaca

SEQ ID NO: 18 - DNA, 21 bp, Artificial Sequence
  oligonucleotide
aagtggttgttgattccgatg

SEQ ID NO: 19 - DNA, 20 bp, Artificial Sequence
  oligonucleotide
tccatgttcaaccagtccaa

SEQ ID NO: 20 - DNA, 18 bp, Artificial Sequence
  oligonucleotide
ctgtcgctggagccactc

SEQ ID NO: 21 - DNA, 20 bp, Artificial Sequence
  oligonucleotide
cttgatgaatgggacagtgg

SEQ ID NO: 22 - DNA, 20 bp, Artificial Sequence
  oligonucleotide
gaccgttctgaggcgttaaa

SEQ ID NO: 23 - DNA, 20 bp, Artificial Sequence
  oligonucleotide
tggaattcttccggatttga

SEQ ID NO: 24 - DNA, 20 bp, Artificial Sequence
  oligonucleotide
ggtttgattgaaggcaggtg

SEQ ID NO: 25 - DNA, 20 bp, Artificial Sequence
  oligonucleotide
agcgagctggtattctccaa

SEQ ID NO: 26 - DNA, 20 bp, Artificial Sequence
  oligonucleotide
acacgctttggacatcatca

SEQ ID NO: 27 - DNA, 80 bp, Artificial Sequence
  oligonucleotide
gacggggtattatgaataaaggatccacgggtaagatttgctgcgctctcttctagttcaagaacggataactcatagac